European Patent Specification EP 2 770 059 B1, published February 12, 2025. Title: Resistance to arthropod pest in tomatoes. Applicant: VILMORIN & CIE. The sequence listing filed with the application follows.

SEQUENCE LISTING (48 sequences)

SEQ ID NO: 1 - DNA, 50 bp, Lycopersicon esculentum
caaaatttgggagagctgaagcagagtttcccactcaaggtaaatgtata

SEQ ID NO: 2 - DNA, 50 bp, Lycopersicon esculentum
agctagtcaaaagtatgccagttgtgtcctgttgcttgtgtatatagttc

SEQ ID NO: 3 - DNA, 50 bp, Lycopersicon esculentum
agtctctaacaatcaagttggtggggatataggctcagacattgagctgg

SEQ ID NO: 4 - DNA, 50 bp, Lycopersicon esculentum
acattcatctgattccgatcaagaagttgatgattacgatgaccttccac

SEQ ID NO: 5 - DNA, 60 bp, Lycopersicon esculentum
gagaaaaagaccattagacaaagaaaaggtgttttgatagctacggagaaaaagagaaag

SEQ ID NO: 6 - DNA, 60 bp, Lycopersicon esculentum
atagagaaaaaaagcaaaacagggagatgaaaggggtctctaatgggagatccattccct

SEQ ID NO: 7 - DNA, 60 bp, Lycopersicon esculentum
taaactaaagtctccttttatttttcatcaataaccttataactaacttaactaaaaaca

SEQ ID NO: 8 - DNA, 60 bp, Lycopersicon esculentum
aggcaatttttatccacaccaaatataaaactaaacttaaatccccattttccaagacat

SEQ ID NO: 9 - DNA, 60 bp, Lycopersicon esculentum
ctgaaggtccagaccacctgtactgcccttctccacacctatgtccagcataaggacact

SEQ ID NO: 10 - DNA, 60 bp, Lycopersicon esculentum
ctaaagctgagtctttgatggaaaaaatgtctgaatgcggggttctgaagtaccctcttc

SEQ ID NO: 11 - DNA, 100 bp, Lycopersicon esculentum
aataatctcccctcctttaaacttggagtatttgaatatcactgtttccgatccacacaaggaaatacaagcatccccctcaattgttcctggcactaat

SEQ ID NO: 12 - DNA, 100 bp, Lycopersicon esculentum
  misc_feature (8)..(8): n is a, c, g, or t
  misc_feature (64)..(64): n is a, c, g, or t
cttatgtnacctatttaattaccacacaaaccaatttacctgattatggaggaaccgatttcantgttcgtagacgctttaaagacattgttactttatc

SEQ ID NO: 13 - DNA, 60 bp, Lycopersicon esculentum
gatgatgaaaaggtggattattcacaagtactttctgcattgcttccttttgttgtggcc

SEQ ID NO: 14 - DNA, 60 bp, Lycopersicon esculentum
tcactgctgttgctgctctttctcacccttcaactttcacatgggtttctaaagatttgt

SEQ ID NO: 15 - DNA, 56 bp, Lycopersicon esculentum
gccggggatagctaacacaccaatattattaatttagagaatcaattatggagatc

SEQ ID NO: 16 - DNA, 60 bp, Lycopersicon esculentum
atgggaactcaaatgatgttcttcacatagttttgttccctttttttcgcatttggtcat

SEQ ID NO: 17 - DNA, 60 bp, Lycopersicon esculentum
aagttgcaagagttgcttttgcctcgcttctcttgttgatgctgatgctatagtaacttc

SEQ ID NO: 18 - DNA, 60 bp, Lycopersicon esculentum
gaatgggttcctaccattgaccaaatgcttctcatgaccagcatagtccttacatatata

SEQ ID NO: 19 - DNA, 60 bp, Lycopersicon esculentum
gtctagtattgttgtaagaatgctggaagaggcatttgtgattataaaagaaacttggca

SEQ ID NO: 20 - DNA, 60 bp, Lycopersicon esculentum
gatataggttataacacagcataaatctatatctaattcacttgaacattacacaagaag

SEQ ID NO: 21 - DNA, 50 bp, Lycopersicon esculentum
ggcttcaatattgactgtaatgaaggagatttctgatacattgtacccaa

SEQ ID NO: 22 - DNA, 50 bp, Lycopersicon esculentum
gcctgtcgtgatttttaatcctaaatggggttttgatgaagagagtagtt

SEQ ID NO: 23 - DNA, 60 bp, Lycopersicon esculentum
tattacggaatctactgtaacgttatcagaagctctgtctgaacttccaggtgaaaggac

SEQ ID NO: 24 - DNA, 60 bp, Lycopersicon esculentum
gaaggtggttctatatccctagatgccttgtcttgcgagaaccatgaaataaagaagatg

SEQ ID NO: 25 - DNA, 60 bp, Lycopersicon esculentum
gtcgcaagatgcgtgagatcatggttaaccaggcacaatcgtgtgatttgaaagacttgg

SEQ ID NO: 26 - DNA, 60 bp, Lycopersicon esculentum
cctgaagttcattcctgaatcaatcggtagagagattgagaaggcaacttcaagcatcta

SEQ ID NO: 27 - DNA, 60 bp, Lycopersicon esculentum
atgggttggttttggagaacatatcgtatgggcagcttcaggcgctttcagctgtgcctg

SEQ ID NO: 28 - DNA, 60 bp, Lycopersicon esculentum
agatagtcactctttgttgactgaggaaagaggcggggaaggtagtgggagtggttcata

SEQ ID NO: 29 - DNA, 60 bp, Lycopersicon esculentum
ttactcttcggtgtttgaggatcttgttgcagagggttttttgagcccaaattcaaaaac

SEQ ID NO: 30 - DNA, 60 bp, Lycopersicon esculentum
ctttgcgttgaaacaccgatgggttctgatgtttttgcgttgagggaaattggggtagcc

SEQ ID NO: 31 - DNA, 60 bp, Lycopersicon esculentum
agttccaattcacgaaatcgaagccttccaactctcatccacgcttggtgattgcaaagg

SEQ ID NO: 32 - DNA, 60 bp, Lycopersicon esculentum
cttggggaccggcgataatggtgactttgaacattttacagctacacctaacaagatttt

SEQ ID NO: 33 - DNA, 50 bp, Lycopersicon esculentum
tttttacttttaaattttgctgtttgtgaagtagggatatgaataaaatt

SEQ ID NO: 34 - DNA, 50 bp, Lycopersicon esculentum
ttggtcccttcttgtacaataggaatgtaagaactagcatatgagggatc

SEQ ID NO: 35 - DNA, 50 bp, Lycopersicon esculentum
aagagggcaaaaaatggctgtagcactcttggggagtatttccttttcct

SEQ ID NO: 36 - DNA, 50 bp, Lycopersicon esculentum
ctccatgccttctatatcttccccttctctccaacaccctttcaacttca

SEQ ID NO: 37 - DNA, 50 bp, Lycopersicon esculentum
aacgccagcaatggaaaagcaacttgagatcgcgtccacagttggtgcat

SEQ ID NO: 38 - DNA, 50 bp, Lycopersicon esculentum
ggttgctaaatccaaccagcccaatgaagtaggtgattttggtggtagtt

SEQ ID NO: 39 - DNA, 50 bp, Lycopersicon esculentum
ggcgcctagaactgcttcttcttttcttgtgacgcgaacttctgtctctt

SEQ ID NO: 40 - DNA, 50 bp, Lycopersicon esculentum
tctcatccaaccactcactgctggaatctgtattacgatcttccttgcta

SEQ ID NO: 41 - DNA, 50 bp, Lycopersicon esculentum
atgttaactgaaattgcatacatccacgttaacaggaaaacatcgtagtc

SEQ ID NO: 42 - DNA, 50 bp, Lycopersicon esculentum
cttctagcaagaactttttaccctgtaatttgaaatccaacaaacccaga

SEQ ID NO: 43 - DNA, 60 bp, Lycopersicon esculentum
aaaccccaatttctccggccgatcagttctcctctttgttgatctcatttttcgattctc

SEQ ID NO: 44 - DNA, 60 bp, Lycopersicon esculentum
gatcactttacagatccgatttcgagtcacttccgaatcggatccgggtcagatggcggc

SEQ ID NO: 45 - DNA, 60 bp, Lycopersicon esculentum
ctagacagtagtgaccaaactcttggtgttccgcgtaagttttagagtataataaaccca

SEQ ID NO: 46 - DNA, 60 bp, Lycopersicon esculentum
aggactcgaaaaacattagctcagatgatgatgaccttgtgtaaattttcgtattggtat

SEQ ID NO: 47 - DNA, 60 bp, Lycopersicon esculentum
ctctagcccatcctttatacacagaagggcgcagccacatcgggagttcctggacgaaca

SEQ ID NO: 48 - DNA, 60 bp, Lycopersicon esculentum
agcatggagtcaagtttttgctgaatcttctgttatttaaaattgatagagacttaccac